European Patent Application EP 4 653 540 A1, published November 26, 2025. Title: フラクトシル化マルチトールおよびその製造方法. Applicant: 京都府公立大学法人. The sequence listing filed with the application follows.

SEQUENCE LISTING (1 sequence)

SEQ ID NO: 1 - protein, 654 aa, Aspergillus fijiensis
MKLTTTTLALATGAAAAEASYHLDTTAPPPTNLSTLPNNTLFHVWRPRAHILPAEGQIGDPCAHYTDPSTGLFHVGFLHDGDGIAGATTANLATYTDTSDNGSFLIQPGGKNDPVAVFDGAVIPVGVNNTPTLLYTSVSFLPIHWSIPYTRGSETQSLAVARDGGRRFDKLDQGPVIADHPFAVDVTAFRDPFVFRSAKLDVLLSLDEEVARNETAVQQAVDGWTEKNAPWYVAVSGGVHGVGPAQFLYRQNGGNASEFQYWEYLGEWWQEATNSSWGDEGTWAGRWGFNFETGNVLFLTEEGHDPQTGEVFVTLGTEGSGLPIVPQVSSIHDMLWAAGEVGVGSEQEGAKVEFSPSMAGFLDWGFSAYAAAGKVLPASSAVSKTSGVEVDRYVSFVWLTGDQYEQADGFPTAQQGWTGSLLLPRELKVQTVENVVDNELVREEGVSWVVGESDNQTARLRTLGITIARETKAALLANGSVTAEEDRTLQTAAVVPFAQSPSSKFFVLTAQLEFPASARSSPLQSGFEILASELERTAIYYQFSNESLVVDRSQTSAAAPTNPGLDSFTESGKLRLFDVIENGQEQVETLDLTVVVDNAVVEVYANGRFALSTWARSWYDNSTQIRFFHNGEGEVQFRNVSVSEGLYNAWPERN